European Patent Application EP 4 464 773 A1, published November 20, 2024. Title: Modified Bacteria with Anti-Tumor Activity. Applicant: SHENZHEN INSTITUTES OF ADVANCED TECHNOLOGY. The sequence listing filed with the application follows.

SEQUENCE LISTING (39 sequences)

SEQ ID NO: 1 - DNA, 3977 bp, synthetic construct
  source 1..3977: mol_type = other DNA
ttcacagaaaagtgttgcccccttccatggcggaagggggacaaaggtgaatttgtcctactcaggagagcgttcaccgacaaacaacagataaaacgaaaggcccagtctttcgactgagcctttcgttttatttgatgcactagtgccgatcatattcaataacccttaatataacttcgtataatgtatgctatacgaagttattaggtctgaagaggagtttacgtcccatatggagtcccgctcagaagaactcgtcaagaaggcgatagaaggcgatgcgctgcgaatcgggagcggcgataccgtaaagcacgaggaagcggtcagcccattcgccgccaagctcttcagcaatatcacgggtagccaacgctatgtcctgatagcggtccgccacacccagccggccacagtcgatgaatccagaaaagcggccattttccaccatgatattcggcaagcaggcatcgccatgggtcacgacgagatcctcgccgtcgggcatgcgcgccttgagcctggcgaacagttcggccggcgcgagcccctgatgctcttcgtccagatcatcctgatcgacaagaccggcttccatccgagtacgtgctcgctcgatgcgatgtttcgcttggtggtcgaatgggcaggtagccggatcaagcgtatgcagccgccgcattgcatcagccatgatggatactttctcggcaggagcaaggtgagatgacaggagatcctgccccggcacttcgcccaatagcagccagtcccttcccgcttcagtgacaacgtcgagcacagctgcgcaaggaacgcccgtcgtggccagccacgatagccgcgctgcctcgtcctgcagttcattcagggcaccggacaggtcggtcttgacaaaaagaaccgggcgcccctgcgctgacagccggaacacggcggcatcagagcagccgattgtctgttgtgcccagtcatagccgaatagcctctccacccaagcggccggagaacctgcgtgcaatccatcttgttcaatcatgcgaaacgatcctcatcctgtctcttgatcagatcctgatcccctgcgccatcagatccttggcggcaagaaagccatccagtttactttgcagggcttcccaaccttaccagagggcgccccagctggcaattccgacgtcattgcgttgctagccaagcttaggatccggaacccttaatataacttcgtataatgtatgctatacgaagttattaggtccctcgaagaggttcactagctatctagagcttggactcctgttgatagatccagtaatgacctcagaactccatctggatttgttcagaacgctcggttgccgccgggcgttttttattggtgagaatccaagcccgggaaacgggatcctgatcttgatcaggctgtgggtcaggccactcttggcatcgacaccaatgtgggccttcatgccaaagtgccactgattgcctttcttggtctgatgcatctccggatcgcgttgctgctctttgttcttggtcgagctgggtgcctcaatgatggtggcatcgaccaaggtgccttgagtcatcatgacgcctgcttcggccagccagcgattgatggtcttgaacaattggcgggccagttgatgctgctccagcaggtggcggaaattcatgatggtggtgcggtccggcaaggcgctatccagggataaccgggcaaacagacgcatggaggcgatttcgtacagagcatcttccatcgcgccatcgctcaggttgtaccaatgctgcatgcagtgaatgcgtagcatggtttccagcggataaggtcgccggccattaccagccttggggtaaaacggctcgatgacttccaccatgttttgccatggcagaatctgctccatgcgggacaagaaaatctcttttctggtctgacggcgcttactgctgaattcactgtcggcgaaggtaagttgatgactcatgatgaaccctgttctatggctccagatgacaaacatgatctcatatcagggacttgttcgcaccttccttagcacgttaattatctatcgtgtatatggaggggatctagaatgaaaaaaataatgctagtttttattacacttatattagttagtctaccaattgcgcaacaaactgaagcaaaggatgcatctgcattcaataaagaaaattcaatttcatccatggcaccaccagcatctccgcctgcaagtcctaagacgccaatcgaaaagaaacacgcggatgaaatcgataagtatatacaaggattggactacaataaaaacaatgtattagtataccacggagatgcagtgacaaatgtgccgccaagaaaaggttacaaagatggaaatgaatatattgttgtggagaaaaagaagaaatccatcaatcaaaataatgcagacattcaagttgtgaatgcaatttcgagcctaacctatccaggtgctctcgtaaaagcgaattcggaattagtagaaaatcaaccagatgttctccctgtaaaacgtgattcattaacactcagcattgatttgccaggtatgactaatcaagacaataaaatcgttgtaaaaaatgccactaaatcaaacgttaacaacgcagtaaatacattagtggaaagatggaatgaaaaatatgctcaagcttatccaaatgtaagtgcaaaaattgattatgatgacgaaatggcttacagtgaatcacaattaattgcgaaatttggtacagcatttaaagctgtaaataatagcttgaatgtaaacttcggcgcaatcagtgaagggaaaatgcaagaagaagtcattagttttaaacaaatttactataacgtgaatgttaatgaacctacaagaccttccagatttttcggcaaagctgttactaaagagcagttgcaagcgcttggagtgaatgcagaaaatcctcctgcatatatctcaagtgtggcgtatggccgtcaagtttatttgaaattatcaactaattcccatagtactaaagtaaaagctgcttttgatgctgccgtaagcggaaaatctgtctcaggtgatgtagaactaacaaatatcatcaaaaattcttccttcaaagccgtaatttacggaggttccgcaaaagatgaagttcaaatcatcgacggcaacctcggagacttacgagatattttgaaaaaaggcgctacttttaatcgagaaacaccaggagttcccattgcttatacaacaaacttcctaaaagacaatgaattagctgttattaaaaacaactcagaatatattgaaacaacttcaaaagcttatacagatggaaaaattaacatcgatcactctggaggatacgttgctcaattcaacatttcttgggatgaagtaaattatgatcctgaaggtaacgaaattgttcaacataaaaactggagcgaaaacaataaaagtaagctagctcatttcacatcgtccatctatttgccaggtaacgcgagaaatattaatgtttacgctaaagaatgcactggtttagcttgggaatggtggagaacggtaattgatgaccggaacttaccacttgtgaaaaatagaaatatctccatctggggcaccacgctttatccgaaatatagtaataaagtagataatccaatcgaataagtcgacctcgaggactagtgaacctcttcgagggacctaataacttcgtatagcatacattatacgaagttatattaagggttattgaatatgatcggctcgagattacttcgcattgcaatcagctacggactcaagcttacgtcaggtcatacgatgaaggcgataagtcgcgtaagttgctagcccacgcggctcaccttcacgggtgggcctttcttcggtgtttcaatctcgattaacaggtaacgcaaaattgctgtgtacgtcaga

SEQ ID NO: 2 - DNA, 2716 bp, synthetic construct
  source 1..2716: mol_type = other DNA
ttggtttcagtgaatcccgttatcagcagttttttgatgaggtgtagtctatttgtcctactcaggagagcgttcaccgacaaacaacagataaaacgaaaggcccagtctttcgactgagcctttcgttttatttgatgcactagtgccgatcatattcaataacccttaatataacttcgtataatgtatgctatacgaagttattaggtctgaagaggagtttacgtcccatatggagtcccgcttacgccccgccctgccactcatcgcagtactgttgtaattcattaagcattctgccgacatggaagccatcacagacggcatgatgaacctgaatcgccagcggcatcagcaccttgtcgccttgcgtataatatttgcccatggtgaaaacgggggcgaagaagttgtccatattggccacgtttaaatcaaaactggtgaaactcacccagggattggctgagacgaaaaacatattctcaataaaccctttagggaaataggccaggttttcaccgtaacacgccacatcttgcgaatatatgtgtagaaactgccggaaatcgtcgtggtattcactccagagcgatgaaaacgtttcagtttgctcatggaaaacggtgtaacaagggtgaacactatcccatatcaccagctcaccgtctttcattgccatacgaaattccggatgagcattcatcaggcgggcaagaatgtgaataaaggccggataaaacttgtgcttatttttctttacggtctttaaaaaggccgtaatatccagctgaacggtctggttataggtacattgagcaactgactgaaatgcctcaaaatgttctttacgatgccattgggatatatcaacggtggtatatccagtgatttttttctccatgcgaaacgatcctcatcctgtctcttgatcagatcctgatcccctgcgccatcagatccttggcggcaagaaagccatccagtttactttgcagggcttcccaaccttaccagagggcgccccagctggcaattccgacgtcattgcgttgctagccaagcttaggatccggaacccttaatataacttcgtataatgtatgctatacgaagttattaggtccctcgaagaggttcactagctatctagagcttggactcctgttgatagatccagtaatgacctcagaactccatctggatttgttcagaacgctcggttgccgccgggcgttttttattggtgagaatccaagcccgggaaacgggatcctgatcttgatcaaccgaggtcacaacatagtaaaagcgctattggtaatggtacaatcgcgcgtttacacttattcagaacgatttttttcaggagggcctacttgtcacacaggacggtaatgtcgtgcccggttattgagctgacacagcaacttattcgtcgcccctccctgagtccggatgacgcaggctgtcaggcattaatgattgaacgcctgcgtaaaatcggttttaccattgagcatatggattttggcgacacgcaaaatttttgggcatggcgtgggcgtggcgaaacgctggcgttcgccgggcatactgacgtcgtaccggctggcgatgtcgatcgctggatcaatccgccgtttgagcctacgattcgcgacggaatgttgttcggtcgcggcgcggcggatatgaaaggttcactggcggccatggtggtggctgctgaacgttttgttgcgcagcatcctcatcaccggggccgcctcgcatttttgattacctctgatgaggaagccagcgcaaaaaatggcaccgtaaaggtggttgaagcgctgatggcccgtaacgagcggctggattactgtctggtcggcgaaccttccagtactgaaattgtgggcgatgtcgtcaaaaacgggcgtcgcggttctctcacctgtaacctcactatccatggcgttcaggggcacgtcgcctatccgcatctggcggataaccctgttcatcgcgccgcgccttttcttaatgaactggtcgctatcgagtgggatcggggcaatgactttttcccggccaccagtatgcaggtagccaatatccaggcaggcaccggcagcaataatgtcattcccggcgaactgttcgtgcagtttaacttccgtttcagcacggaactgaccgatgagatgatcaaagagcgggtacatgcgctgcttgaaaagcatcagctacgctataccgtagactggtggctttccgggcagccgttcctgaccgcacgcggcaagctggtggacgcggtggtaaacgccattgagcactataatgaaattaaaccgcaattactgacgacgggcggtacgtccgacggacgttttatcgcccgtatgggagcgcaggtggtagaactggggccggtgaacgccaccattcataaaattaatgaatgtgtgaatgccgccgatctccagctactggcccgtatgtatcaacgcattatggaacagctcgtcgcccatcaccatcaccatcactaagattacttcgcattgcaatcagctacggactcaagcttacgtcaggtcatacgatgaaggcgataagtcgcgtaagttgctagcccacgcggctcaccttcacgggtgggcctttcttcgtgagcgttccggtaagaggaaataagcatggactggctggcaaaatattg

SEQ ID NO: 3 - DNA, 1236 bp, synthetic construct
  source 1..1236: mol_type = other DNA
ttattcgattggattatctactttattactatatttcggataaagcgtggctagtgaacctcttcgagggacctaataacttcgtatagcatacattatacgaagttatattaagggttccggatcctaagcttggctagcaacgcaatgacgtcggaattgccagctggggcgccctctggtaaggttgggaagccctgcaaagtaaactggatggctttcttgccgccaaggatctgatggcgcaggggatcaggatctgatcaagagacaggatgaggatcgtttcgcatgattgaacaagatggattgcacgcaggttctccggccgcttgggtggagaggctattcggctatgactgggcacaacagacaatcggctgctctgatgccgccgtgttccggctgtcagcgcaggggcgcccggttctttttgtcaagaccgacctgtccggtgccctgaatgaactgcaggacgaggcagcgcggctatcgtggctggccacgacgggcgttccttgcgcagctgtgctcgacgttgtcactgaagcgggaagggactggctgctattgggcgaagtgccggggcaggatctcctgtcatctcaccttgctcctgccgagaaagtatccatcatggctgatgcaatgcggcggctgcatacgcttgatccggctacctgcccattcgaccaccaagcgaaacatcgcatcgagcgagcacgtactcggatggaagccggtcttgtcgatcaggatgatctggacgaagagcatcaggggctcgcgccggccgaactgttcgccaggctcaaggcgcgcatgcccgacggcgaggatctcgtcgtgacccatggcgatgcctgcttgccgaatatcatggtggaaaatggccgcttttctggattcatcgactgtggccggctgggtgtggcggaccgctatcaggacatagcgttggctacccgtgatattgctgaagagcttggcggcgaatgggctgaccgcttcctcgtgctttacggtatcgccgctcccgattcgcagcgcatcgccttctatcgccttcttgacgagttcttctgagcgggactccatatgggacgtaaactcctcttcagacctaataacttcgtatagcatacattatacgaagttatattaagggttattgaatatgatcggcggtagactaactaatataagtgtaataaaaactagcattatttttttcat

SEQ ID NO: 4 - DNA, 3065 bp, synthetic construct
  source 1..3065: mol_type = other DNA
caatattttgccagccagtccatgcttatttcctcttaccggaacgctcaatttgtcctactcaggagagcgttcaccgacaaacaacagataaaacgaaaggcccagtctttcgactgagcctttcgttttatttgatgcactagtgccgatcatattcaataacccttaatataacttcgtataatgtatgctatacgaagttattaggtctgaagaggagtttacgtcccatatggagtcccgctcagaagaactcgtcaagaaggcgatagaaggcgatgcgctgcgaatcgggagcggcgataccgtaaagcacgaggaagcggtcagcccattcgccgccaagctcttcagcaatatcacgggtagccaacgctatgtcctgatagcggtccgccacacccagccggccacagtcgatgaatccagaaaagcggccattttccaccatgatattcggcaagcaggcatcgccatgggtcacgacgagatcctcgccgtcgggcatgcgcgccttgagcctggcgaacagttcggccggcgcgagcccctgatgctcttcgtccagatcatcctgatcgacaagaccggcttccatccgagtacgtgctcgctcgatgcgatgtttcgcttggtggtcgaatgggcaggtagccggatcaagcgtatgcagccgccgcattgcatcagccatgatggatactttctcggcaggagcaaggtgagatgacaggagatcctgccccggcacttcgcccaatagcagccagtcccttcccgcttcagtgacaacgtcgagcacagctgcgcaaggaacgcccgtcgtggccagccacgatagccgcgctgcctcgtcctgcagttcattcagggcaccggacaggtcggtcttgacaaaaagaaccgggcgcccctgcgctgacagccggaacacggcggcatcagagcagccgattgtctgttgtgcccagtcatagccgaatagcctctccacccaagcggccggagaacctgcgtgcaatccatcttgttcaatcatgcgaaacgatcctcatcctgtctcttgatcagatcctgatcccctgcgccatcagatccttggcggcaagaaagccatccagtttactttgcagggcttcccaaccttaccagagggcgccccagctggcaattccgacgtcattgcgttgctagccaagcttaggatccggaacccttaatataacttcgtataatgtatgctatacgaagttattaggtccctcgaagaggttcactagctatctagagcttggactcctgttgatagatccagtaatgacctcagaactccatctggatttgttcagaacgctcggttgccgccgggcgttttttattggtgagaatccaagcccgggaaacgggatcctgatcttgatcaggaacatggcattgattatcgttttcacgattaccgtgtggatggcatagacctccctcttcttaatacctttattgccgaactcggctggcagcctttactgaatacgcgcggcacaacatggcgcaaactggatgaaggccaccgcagcgggattaccgatgccgactccgccgctgctctcatggttgaacagccggcaatcatcaaacgcccattgctctgcgcgcccgggaagcctatgctgcttggtttcagtgaatcccgttatcagcagttttttgatgaggtgtagtctggcctacttgtcacacaggacggtaatgtcgtgcccggttattgagctgacacagcaacttattcgtcgcccctccctgagtccggatgacgcaggctgtcaggcattaatgattgaacgcctgcgtaaaatcggttttaccattgagcatatggattttggcgacacgcaaaatttttgggcatggcgtgggcgtggcgaaacgctggcgttcgccgggcatactgacgtcgtaccggctggcgatgtcgatcgctggatcaatccgccgtttgagcctacgattcgcgacggaatgttgttcggtcgcggcgcggcggatatgaaaggttcactggcggccatggtggtggctgctgaacgttttgttgcgcagcatcctcatcaccggggccgcctcgcatttttgattacctctgatgaggaagccagcgcaaaaaatggcaccgtaaaggtggttgaagcgctgatggcccgtaacgagcggctggattactgtctggtcggcgaaccttccagtactgaaattgtgggcgatgtcgtcaaaaacgggcgtcgcggttctctcacctgtaacctcactatccatggcgttcaggggcacgtcgcctatccgcatctggcggataaccctgttcatcgcgccgcgccttttcttaatgaactggtcgctatcgagtgggatcggggcaatgactttttcccggccaccagtatgcaggtagccaatatccaggcaggcaccggcagcaataatgtcattcccggcgaactgttcgtgcagtttaacttccgtttcagcacggaactgaccgatgagatgatcaaagagcgggtacatgcgctgcttgaaaagcatcagctacgctataccgtagactggtggctttccgggcagccgttcctgaccgcacgcggcaagctggtggacgcggtggtaaacgccattgagcactataatgaaattaaaccgcaattactgacgacgggcggtacgtccgacggacgttttatcgcccgtatgggagcgcaggtggtagaactggggccggtgaacgccaccattcataaaattaatgaatgtgtgaatgccgccgatctccagctactggcccgtatgtatcaacgcattatggaacagctcgtcgcccatcaccatcaccatcactaagattacttcgcattgcaatcagctacggactcaagcttacgtcaggtcatacgatgaaggcgataagtcgcgtaagttgctagcccacgcggctcaccttcacgggtgggcctttcttcgagactacacctcatcaaaaaactgctgataacgggattcactgaaaccaa

SEQ ID NO: 5 - DNA, 3142 bp, synthetic construct
  source 1..3142: mol_type = other DNA
gataatgtattcacaggttgctccgggcttgaaaaagttaaatgacatccatttgtcctactcaggagagcgttcaccgacaaacaacagataaaacgaaaggcccagtctttcgactgagcctttcgttttatttgatgcactagtgccgatcatattcaataacccttaatataacttcgtataatgtatgctatacgaagttattaggtctgaagaggagtttacgtcccatatggagtcccgccttatttgccgactaccttggtgatctcgcctttcacgtagtggacaaattcttccaactgatctgcgcgcgaggccaagcgatcttcttcttgtccaagataagcctgtctagcttcaagtatgacgggctgatactgggccggcaggcgctccattgcccagtcggcagcgacatccttcggcgcgattttgccggttactgcgctgtaccaaatgcgggacaacgtaagcactacatttcgctcatcgccagcccagtcgggcggcgagttccatagcgttaaggtttcatttagcgcctcaaatagatcctgttcaggaaccggatcaaagagttcctccgccgctggacctaccaaggcaacgctatgttctcttgcttttgtcagcaagatagccagatcaatgtcgatcgtggctggctcgaagatacctgcaagaatgtcattgcgctgccattctccaaattgcagttcgcgcttagctggataacgccacggaatgatgtcgtcgtgcacaacaatggtgacttctacagcgcggagaatctcgctctctccaggggaagccgaagtttccaaaaggtcgttgatcaaagctcgccgcgttgtttcatcaagccttacggtcaccgtaaccagcaaatcaatatcactgtgtggcttcaggccgccatccactgcggagccgtacaaatgtacggccagcaacgtcggttcgagatggcgctcgatgacgccaactacctctgatagttgagtcgatacttcggcgatcaccgcttccctcatgacattgcactccaccgctgatgacatcagtcgatcatagcacgatcaacggcactgttgcaaatagtcggtggtgataaacttatcatccccttttgctgatggagctgcacatgaactcgagacgtcattgcgttgctagccaagcttaggatccggaacccttaatataacttcgtataatgtatgctatacgaagttattaggtccctcgaagaggttcactagctatctagagcttggactcctgttgatagatccagtaatgacctcagaactccatctggatttgttcagaacgctcggttgccgccgggcgttttttattggtgagaatccaagccttatcgctgtcggttgattcaggattatatcagcgggatgactgacctttacgcatgggatgaatatcggcgtttgatggcggtcgaacagtaaatggacttttgtaaagatggacaataaatttttactttttccagaaactttattccggaacttcgcgttataaaatgaatctgacgtacacagcaattttgcgttacctgttaatcgagattgaaacacatgaaaaaaaccacattagcaatgagtgcactggctctgagtttaggtttggcattgtcgcctctgtctgccacggcggctgaaacgtcctcttcagcaatgactgcccagcagatgccaagcctggcaccgatgctcgaaaaagtgatgccatcggtggtcagtattaatgttgaaggtagcaccacggtgaatacgccgcgtatgccgcgtaatttccagcagttctttggcgatgactccccgttctgccaggacggttctccgttccagaattctccgttctgccagggcggcggtaacggcggcaacggcggtcaacaacagaaattcatggcgctgggctccggcgtaattattgacgccgcgaagggctacgtcgtcaccaacaaccacgtggttgataacgccagcgtgattaaagtacagcttagcgatgggcgtaaattcgatgctaaagtggtgggcaaagatccgcgttctgatatcgcgctgattcaaattcagaatccgaagaacctgacggcgattaagctggcggactccgacgcgctgcgcgtgggggattataccgtcgctattggtaacccgtttggtctgggcgaaacggtgacgtcaggtatcgtttcggcgctggggcgtagcggcctgaacgtagaaaattacgagaactttattcagaccgacgccgcgattaaccgtggtaactccggcggcgcgctggtgaacctgaacggtgagctgatcggtattaacaccgcgattctggcgccggacggcggcaacatcggtatcggcttcgctatccccagtaacatggtgaaaaacctgacgtcgcagatggtggaatacggccaggtgaaacgcggcgaactggggatcatggggactgagctgaattccgaattggcgaaagcgatgaaagtcgacgcccagcgaggcgcgttcgtcagccaggtgatgccgaattcgtccgcggcgaaagcgggtatcaaagccggggatgtcattacctcgctgaacggtaaaccgatcagcagctttgcggcgctgcgcgctcaggtcggcactatgccggtcggcagcaaaatcagcctcggtctgctgcgtgaaggtaaagcgattacggtgaatctggaactgcagcagagcagccagagtcaggttgattccagcaccatcttcagcgggattgaaggcgctgaaatgagcaataaaggccaggataaaggcgttgtggtgagcagcgtgaaagcgaactcacccgccgcgcaaattggcctcaaaaaaggcgatgtgattatcggcgctaaccagcagccggtgaaaaatatcgccgagctgcgtaagattctcgacagcaagccgtcggttctggcgctgaatattcagcgtggtgatagttctatttatttgctgatgcagtaagaagtcgcgtaagttgctagcccacgcggctcaccttcacgggtgggcctttcttcgtatactaagttgaacgaaacgggaaggcgaaaaggtaaaaagttcctttt

SEQ ID NO: 6 - DNA, 1236 bp, synthetic construct
  source 1..1236: mol_type = other DNA
aggtagtacagggtttgtcagcataaagcctctcttacgagaggctttatgccgatcatattcaataacccttaatataacttcgtataatgtatgctatacgaagttattaggtctgaagaggagtttacgtcccatatggagtcccgctcagaagaactcgtcaagaaggcgatagaaggcgatgcgctgcgaatcgggagcggcgataccgtaaagcacgaggaagcggtcagcccattcgccgccaagctcttcagcaatatcacgggtagccaacgctatgtcctgatagcggtccgccacacccagccggccacagtcgatgaatccagaaaagcggccattttccaccatgatattcggcaagcaggcatcgccatgggtcacgacgagatcctcgccgtcgggcatgcgcgccttgagcctggcgaacagttcggccggcgcgagcccctgatgctcttcgtccagatcatcctgatcgacaagaccggcttccatccgagtacgtgctcgctcgatgcgatgtttcgcttggtggtcgaatgggcaggtagccggatcaagcgtatgcagccgccgcattgcatcagccatgatggatactttctcggcaggagcaaggtgagatgacaggagatcctgccccggcacttcgcccaatagcagccagtcccttcccgcttcagtgacaacgtcgagcacagctgcgcaaggaacgcccgtcgtggccagccacgatagccgcgctgcctcgtcctgcagttcattcagggcaccggacaggtcggtcttgacaaaaagaaccgggcgcccctgcgctgacagccggaacacggcggcatcagagcagccgattgtctgttgtgcccagtcatagccgaatagcctctccacccaagcggccggagaacctgcgtgcaatccatcttgttcaatcatgcgaaacgatcctcatcctgtctcttgatcagatcctgatcccctgcgccatcagatccttggcggcaagaaagccatccagtttactttgcagggcttcccaaccttaccagagggcgccccagctggcaattccgacgtcattgcgttgctagccaagcttaggatccggaacccttaatataacttcgtataatgtatgctatacgaagttattaggtccctcgaagaggttcactaggcttttccagggtctgctgacgcgaaaaggaattgtgaatagtgtagcga

SEQ ID NO: 7 - DNA, 1236 bp, synthetic construct
  source 1..1236: mol_type = other DNA
cggacaaaaaaatggcgcacgatgtgcgccattttatattgtgcgtcaaagccgatcatattcaataacccttaatataacttcgtataatgtatgctatacgaagttattaggtctgaagaggagtttacgtcccatatggagtcccgctcagaagaactcgtcaagaaggcgatagaaggcgatgcgctgcgaatcgggagcggcgataccgtaaagcacgaggaagcggtcagcccattcgccgccaagctcttcagcaatatcacgggtagccaacgctatgtcctgatagcggtccgccacacccagccggccacagtcgatgaatccagaaaagcggccattttccaccatgatattcggcaagcaggcatcgccatgggtcacgacgagatcctcgccgtcgggcatgcgcgccttgagcctggcgaacagttcggccggcgcgagcccctgatgctcttcgtccagatcatcctgatcgacaagaccggcttccatccgagtacgtgctcgctcgatgcgatgtttcgcttggtggtcgaatgggcaggtagccggatcaagcgtatgcagccgccgcattgcatcagccatgatggatactttctcggcaggagcaaggtgagatgacaggagatcctgccccggcacttcgcccaatagcagccagtcccttcccgcttcagtgacaacgtcgagcacagctgcgcaaggaacgcccgtcgtggccagccacgatagccgcgctgcctcgtcctgcagttcattcagggcaccggacaggtcggtcttgacaaaaagaaccgggcgcccctgcgctgacagccggaacacggcggcatcagagcagccgattgtctgttgtgcccagtcatagccgaatagcctctccacccaagcggccggagaacctgcgtgcaatccatcttgttcaatcatgcgaaacgatcctcatcctgtctcttgatcagatcctgatcccctgcgccatcagatccttggcggcaagaaagccatccagtttactttgcagggcttcccaaccttaccagagggcgccccagctggcaattccgacgtcattgcgttgctagccaagcttaggatccggaacccttaatataacttcgtataatgtatgctatacgaagttattaggtccctcgaagaggttcactagtattaataccctctagattgagttaatctccatgtagcgttacaagtatt

SEQ ID NO: 8 - DNA, 1236 bp, synthetic construct
  source 1..1236: mol_type = other DNA
gctttcgctgccttgattgtgtaccacgtgtcggtgaatcaatcgccggagccgatcatattcaataacccttaatataacttcgtataatgtatgctatacgaagttattaggtctgaagaggagtttacgtcccatatggagtcccgctcagaagaactcgtcaagaaggcgatagaaggcgatgcgctgcgaatcgggagcggcgataccgtaaagcacgaggaagcggtcagcccattcgccgccaagctcttcagcaatatcacgggtagccaacgctatgtcctgatagcggtccgccacacccagccggccacagtcgatgaatccagaaaagcggccattttccaccatgatattcggcaagcaggcatcgccatgggtcacgacgagatcctcgccgtcgggcatgcgcgccttgagcctggcgaacagttcggccggcgcgagcccctgatgctcttcgtccagatcatcctgatcgacaagaccggcttccatccgagtacgtgctcgctcgatgcgatgtttcgcttggtggtcgaatgggcaggtagccggatcaagcgtatgcagccgccgcattgcatcagccatgatggatactttctcggcaggagcaaggtgagatgacaggagatcctgccccggcacttcgcccaatagcagccagtcccttcccgcttcagtgacaacgtcgagcacagctgcgcaaggaacgcccgtcgtggccagccacgatagccgcgctgcctcgtcctgcagttcattcagggcaccggacaggtcggtcttgacaaaaagaaccgggcgcccctgcgctgacagccggaacacggcggcatcagagcagccgattgtctgttgtgcccagtcatagccgaatagcctctccacccaagcggccggagaacctgcgtgcaatccatcttgttcaatcatgcgaaacgatcctcatcctgtctcttgatcagatcctgatcccctgcgccatcagatccttggcggcaagaaagccatccagtttactttgcagggcttcccaaccttaccagagggcgccccagctggcaattccgacgtcattgcgttgctagccaagcttaggatccggaacccttaatataacttcgtataatgtatgctatacgaagttattaggtccctcgaagaggttcactagatcaattacaacttgatgttattgggctgttgcccacggtttctcaccgt

SEQ ID NO: 9 - DNA, 6750 bp, synthetic construct
  source 1..6750: mol_type = other DNA
catggtcatagctgtttcctttaatgcccatggcgtttaccaatgcttaatcagtgaggcacctatctcagcgatctgtctatttcgttcatccatagttgcctgactccccgtcgtgtagataactacgatacgggagggcttaccatctggccccagtgctgcaatgataccgcgacttccacgctcaccggctccagatttatcagcaataaaccagccagccggaagggccgagcgcagaagtggtcctgcaactttatccgcctccatccagtctattaattgttgccgggaagctagagtaagtagttcgccagttaatagtttgcgcaacgttgttgccattgctacaggcatcgtggtgtcacgctcgtcgtttggtatggcttcattcagctccggttcccaacgatcaaggcgagttacatgatcccccatgttgtgcaaaaaagcggttagctccttcggtcctccgatcgttgtcagaagtaagttggccgcagtgttatcactcatggttatggcagcactgcataattctcttactgtcatgccatccgtaagatgcttttctgtgactggtgagtactcaaccaagtcattctgagaatagtgtatgcggcgaccgagttgctcttgcccggcgtcaatacgggataataccgcgccacatagcagaactttaaaagtgctcatcattggaaaacgttcttcggggcgaaaactctcaaggatcttaccgctgttgagatccagttcgatgtaacccactcgtgcacccaactgatcttcagcatcttttactttcaccagcgtttctgggtgagcaaaaacaggaaggcaaaatgccgcaaaaaagggaataagggcgacacggaaatgttgaatactcatactcttcctttttcaatattattgaagcatttatcagggttattgtctcatgagcggatacatatttgaatgtatttagaaaaataaacaaataggggttccgcgcacatttccccgaaaagtgccacctgacgtctaagaaaccattattatcatgacattaacctataaaaataggcgtatcacgaggcccttaggccaaataggccgttcagatccttccgtatttagccagtatgttctctagtgtggttcgttgtttttgcgtgagccatgagaacgaaccattgagatcatgcttactttgcatgtcactcaaaaattttgcctcaaaactggtgagctgaatttttgcagttaaagcatcgtgtagtgtttttcttagtccgttacgtaggtaggaatctgatgtaatggttgttggtattttgtcaccattcatttttatctggttgttctcaagttcggttacgagatccatttgtctatctagttcaacttggaaaatcaacgtatcagtcgggcggcctcgcttatcaaccaccaatttcatattgctgtaagtgtttaaatctttacttattggtttcaaaacccattggttaagccttttaaactcatggtagttattttcaagcattaacatgaacttaaattcatcaaggctaatctctatatttgccttgtgagttttcttttgtgttagttcttttaataaccactcataaatcctcatagagtatttgttttcaaaagacttaacatgttccagattatattttatgaatttttttaactggaaaagataaggcaatatctcttcactaaaaactaattctaatttttcgcttgagaacttggcatagtttgtccactggaaaatctcaaagcctttaaccaaaggattcctgatttccacagttctcgtcatcagctctctggttgctttagctaatacaccataagcattttccctactgatgttcatcatctgagcgtattggttataagtgaacgataccgtccgttctttccttgtagggttttcaatcgtggggttgagtagtgccacacagcataaaattagcttggtttcatgctccgttaagtcatagcgactaatcgctagttcatttgctttgaaaacaactaattcagacatacatctcaattggtctaggtgattttaatcactataccaattgagatgggctagtcaatgataattactagtccttttcctttgagttgtgggtatctgtaaattctgctagacctttgctggaaaacttgtaaattctgctagaccctctgtaaattccgctagacctttgtgtgttttttttgtttatattcaagtggttataatttatagaataaagaaagaataaaaaaagataaaaagaatagatcccagccctgtgtataactcactactttagtcagttccgcagtattacaaaaggatgtcgcaaacgctgtttgctcctctacaaaacagaccttaaaaccctaaaggcttaagtagcaccctcgcaagctcgggcaaatcgctgaatattccttttgtctccgaccatcaggcacctgagtcgctgtctttttcgtgacattcagttcgctgcgctcacggctctggcagtgaatgggggtaaatggcactacaggcgccttttatggattcatgcaaggaaactacccataatacaagaaaagcccgtcacgggcttctcagggcgttttatggcgggtctgctatgtggtgctatctgactttttgctgttcagcagttcctgccctctgattttccagtctgaccacttcggattatcccgtgacaggtcattcagactggctaatgcacccagtaaggcagcggtatcatcaacaggcttacccgtcttactgtcaagaggacatccggtcagataaccgtcatcttcggctactgtctagggcggcggatttgtcctactcaggagagcgttcaccgacaaacaacagataaaacgaaaggcccagtctttcgactgagcctttcgttttatttgatgcactagtgccgatcatattcaataacccttaatataacttcgtataatgtatgctatacgaagttattaggtctgaagaggagtttacgtcccatatggagtcccgctcagaagaactcgtcaagaaggcgatagaaggcgatgcgctgcgaatcgggagcggcgataccgtaaagcacgaggaagcggtcagcccattcgccgccaagctcttcagcaatatcacgggtagccaacgctatgtcctgatagcggtccgccacacccagccggccacagtcgatgaatccagaaaagcggccattttccaccatgatattcggcaagcaggcatcgccatgggtcacgacgagatcctcgccgtcgggcatgcgcgccttgagcctggcgaacagttcggccggcgcgagcccctgatgctcttcgtccagatcatcctgatcgacaagaccggcttccatccgagtacgtgctcgctcgatgcgatgtttcgcttggtggtcgaatgggcaggtagccggatcaagcgtatgcagccgccgcattgcatcagccatgatggatactttctcggcaggagcaaggtgagatgacaggagatcctgccccggcacttcgcccaatagcagccagtcccttcccgcttcagtgacaacgtcgagcacagctgcgcaaggaacgcccgtcgtggccagccacgatagccgcgctgcctcgtcctgcagttcattcagggcaccggacaggtcggtcttgacaaaaagaaccgggcgcccctgcgctgacagccggaacacggcggcatcagagcagccgattgtctgttgtgcccagtcatagccgaatagcctctccacccaagcggccggagaacctgcgtgcaatccatcttgttcaatcatgcgaaacgatcctcatcctgtctcttgatcagatcctgatcccctgcgccatcagatccttggcggcaagaaagccatccagtttactttgcagggcttcccaaccttaccagagggcgccccagctggcaattccgacgtcattgcgttgctagccaagcttaggatccggaacccttaatataacttcgtataatgtatgctatacgaagttattaggtccctcgaagaggttcactagctatctagagcttggactcctgttgatagatccagtaatgacctcagaactccatctggatttgttcagaacgctcggttgccgccgggcgttttttattggtgagaatccaagcccgggaaacgggatcctgatcttgatcaggctgtgggtcaggccactcttggcatcgacaccaatgtgggccttcatgccaaagtgccactgattgcctttcttggtctgatgcatctccggatcgcgttgctgctctttgttcttggtcgagctgggtgcctcaatgatggtggcatcgaccaaggtgccttgagtcatcatgacgcctgcttcggccagccagcgattgatggtcttgaacaattggcgggccagttgatgctgctccagcaggtggcggaaattcatgatggtggtgcggtccggcaaggcgctatccagggataaccgggcaaacagacgcatggaggcgatttcgtacagagcatcttccatcgcgccatcgctcaggttgtaccaatgctgcatgcagtgaatgcgtagcatggtttccagcggataaggtcgccggccattaccagccttggggtaaaacggctcgatgacttccaccatgttttgccatggcagaatctgctccatgcgggacaagaaaatctcttttctggtctgacggcgcttactgctgaattcactgtcggcgaaggtaagttgatgactcatgatgaaccctgttctatggctccagatgacaaacatgatctcatatcagggacttgttcgcaccttccttagcacgttaattatctatcgtgtatatggaggggatctagaatgaaaaaaataatgctagtttttattacacttatattagttagtctaccaattgcgcaacaaactgaagcaaaggatgcatctgcattcaataaagaaaattcaatttcatccatggcaccaccagcatctccgcctgcaagtcctaagacgccaatcgaaaagaaacacgcggatgaaatcgataagtatatacaaggattggactacaataaaaacaatgtattagtataccacggagatgcagtgacaaatgtgccgccaagaaaaggttacaaagatggaaatgaatatattgttgtggagaaaaagaagaaatccatcaatcaaaataatgcagacattcaagttgtgaatgcaatttcgagcctaacctatccaggtgctctcgtaaaagcgaattcggaattagtagaaaatcaaccagatgttctccctgtaaaacgtgattcattaacactcagcattgatttgccaggtatgactaatcaagacaataaaatcgttgtaaaaaatgccactaaatcaaacgttaacaacgcagtaaatacattagtggaaagatggaatgaaaaatatgctcaagcttatccaaatgtaagtgcaaaaattgattatgatgacgaaatggcttacagtgaatcacaattaattgcgaaatttggtacagcatttaaagctgtaaataatagcttgaatgtaaacttcggcgcaatcagtgaagggaaaatgcaagaagaagtcattagttttaaacaaatttactataacgtgaatgttaatgaacctacaagaccttccagatttttcggcaaagctgttactaaagagcagttgcaagcgcttggagtgaatgcagaaaatcctcctgcatatatctcaagtgtggcgtatggccgtcaagtttatttgaaattatcaactaattcccatagtactaaagtaaaagctgcttttgatgctgccgtaagcggaaaatctgtctcaggtgatgtagaactaacaaatatcatcaaaaattcttccttcaaagccgtaatttacggaggttccgcaaaagatgaagttcaaatcatcgacggcaacctcggagacttacgagatattttgaaaaaaggcgctacttttaatcgagaaacaccaggagttcccattgcttatacaacaaacttcctaaaagacaatgaattagctgttattaaaaacaactcagaatatattgaaacaacttcaaaagcttatacagatggaaaaattaacatcgatcactctggaggatacgttgctcaattcaacatttcttgggatgaagtaaattatgatcctgaaggtaacgaaattgttcaacataaaaactggagcgaaaacaataaaagtaagctagctcatttcacatcgtccatctatttgccaggtaacgcgagaaatattaatgtttacgctaaagaatgcactggtttagcttgggaatggtggagaacggtaattgatgaccggaacttaccacttgtgaaaaatagaaatatctccatctggggcaccacgctttatccgaaatatagtaataaagtagataatccaatcgaataagtcgacctcgaggactagtgaacctcttcgagggacctaataacttcgtatagcatacattatacgaagttatattaagggttattgaatatgatcggctcgagattacttcgcattgcaatcagctacggactcaagcttacgtcaggtcatacgatgaaggcgataagtcgcgtaagttgctagcccacgcggctcaccttcacgggtgggcctttcttcgcgatccacatg

SEQ ID NO: 10 - DNA, 5456 bp, synthetic construct
  source 1..5456: mol_type = other DNA
catggtcatagctgtttcctttaatgcccatggcgtttaccaatgcttaatcagtgaggcacctatctcagcgatctgtctatttcgttcatccatagttgcctgactccccgtcgtgtagataactacgatacgggagggcttaccatctggccccagtgctgcaatgataccgcgacttccacgctcaccggctccagatttatcagcaataaaccagccagccggaagggccgagcgcagaagtggtcctgcaactttatccgcctccatccagtctattaattgttgccgggaagctagagtaagtagttcgccagttaatagtttgcgcaacgttgttgccattgctacaggcatcgtggtgtcacgctcgtcgtttggtatggcttcattcagctccggttcccaacgatcaaggcgagttacatgatcccccatgttgtgcaaaaaagcggttagctccttcggtcctccgatcgttgtcagaagtaagttggccgcagtgttatcactcatggttatggcagcactgcataattctcttactgtcatgccatccgtaagatgcttttctgtgactggtgagtactcaaccaagtcattctgagaatagtgtatgcggcgaccgagttgctcttgcccggcgtcaatacgggataataccgcgccacatagcagaactttaaaagtgctcatcattggaaaacgttcttcggggcgaaaactctcaaggatcttaccgctgttgagatccagttcgatgtaacccactcgtgcacccaactgatcttcagcatcttttactttcaccagcgtttctgggtgagcaaaaacaggaaggcaaaatgccgcaaaaaagggaataagggcgacacggaaatgttgaatactcatactcttcctttttcaatattattgaagcatttatcagggttattgtctcatgagcggatacatatttgaatgtatttagaaaaataaacaaataggggttccgcgcacatttccccgaaaagtgccacctgacgtctaagaaaccattattatcatgacattaacctataaaaataggcgtatcacgaggcccttaggccaaataggccgttcagatccttccgtatttagccagtatgttctctagtgtggttcgttgtttttgcgtgagccatgagaacgaaccattgagatcatgcttactttgcatgtcactcaaaaattttgcctcaaaactggtgagctgaatttttgcagttaaagcatcgtgtagtgtttttcttagtccgttacgtaggtaggaatctgatgtaatggttgttggtattttgtcaccattcatttttatctggttgttctcaagttcggttacgagatccatttgtctatctagttcaacttggaaaatcaacgtatcagtcgggcggcctcgcttatcaaccaccaatttcatattgctgtaagtgtttaaatctttacttattggtttcaaaacccattggttaagccttttaaactcatggtagttattttcaagcattaacatgaacttaaattcatcaaggctaatctctatatttgccttgtgagttttcttttgtgttagttcttttaataaccactcataaatcctcatagagtatttgttttcaaaagacttaacatgttccagattatattttatgaatttttttaactggaaaagataaggcaatatctcttcactaaaaactaattctaatttttcgcttgagaacttggcatagtttgtccactggaaaatctcaaagcctttaaccaaaggattcctgatttccacagttctcgtcatcagctctctggttgctttagctaatacaccataagcattttccctactgatgttcatcatctgagcgtattggttataagtgaacgataccgtccgttctttccttgtagggttttcaatcgtggggttgagtagtgccacacagcataaaattagcttggtttcatgctccgttaagtcatagcgactaatcgctagttcatttgctttgaaaacaactaattcagacatacatctcaattggtctaggtgattttaatcactataccaattgagatgggctagtcaatgataattactagtccttttcctttgagttgtgggtatctgtaaattctgctagacctttgctggaaaacttgtaaattctgctagaccctctgtaaattccgctagacctttgtgtgttttttttgtttatattcaagtggttataatttatagaataaagaaagaataaaaaaagataaaaagaatagatcccagccctgtgtataactcactactttagtcagttccgcagtattacaaaaggatgtcgcaaacgctgtttgctcctctacaaaacagaccttaaaaccctaaaggcttaagtagcaccctcgcaagctcgggcaaatcgctgaatattccttttgtctccgaccatcaggcacctgagtcgctgtctttttcgtgacattcagttcgctgcgctcacggctctggcagtgaatgggggtaaatggcactacaggcgccttttatggattcatgcaaggaaactacccataatacaagaaaagcccgtcacgggcttctcagggcgttttatggcgggtctgctatgtggtgctatctgactttttgctgttcagcagttcctgccctctgattttccagtctgaccacttcggattatcccgtgacaggtcattcagactggctaatgcacccagtaaggcagcggtatcatcaacaggcttacccgtcttactgtcaagaggacatccggtcagataaccgtcatcttcggctactgtctagggcggcggatttgtcctactcaggagagcgttcaccgacaaacaacagataaaacgaaaggcccagtctttcgactgagcctttcgttttatttgatgcactagtgccgatcatattcaataacccttaatataacttcgtataatgtatgctatacgaagttattaggtctgaagaggagtttacgtcccatatggagtcccgcttacgccccgccctgccactcatcgcagtactgttgtaattcattaagcattctgccgacatggaagccatcacagacggcatgatgaacctgaatcgccagcggcatcagcaccttgtcgccttgcgtataatatttgcccatggtgaaaacgggggcgaagaagttgtccatattggccacgtttaaatcaaaactggtgaaactcacccagggattggctgagacgaaaaacatattctcaataaaccctttagggaaataggccaggttttcaccgtaacacgccacatcttgcgaatatatgtgtagaaactgccggaaatcgtcgtggtattcactccagagcgatgaaaacgtttcagtttgctcatggaaaacggtgtaacaagggtgaacactatcccatatcaccagctcaccgtctttcattgccatacgaaattccggatgagcattcatcaggcgggcaagaatgtgaataaaggccggataaaacttgtgcttatttttctttacggtctttaaaaaggccgtaatatccagctgaacggtctggttataggtacattgagcaactgactgaaatgcctcaaaatgttctttacgatgccattgggatatatcaacggtggtatatccagtgatttttttctccattttagcttccttagctcctgaaaatctcgataactcaaaaaatacgcccggtagtgatcttatttcattatggtgaaagttggaacctcttacgtgccgatcagacgtcattgcgttgctagccaagcttaggatccggaacccttaatataacttcgtataatgtatgctatacgaagttattaggtccctcgaagaggttcactagctatctagagcttggactcctgttgatagatccagtaatgacctcagaactccatctggatttgttcagaacgctcggttgccgccgggcgttttttattggtgagaatccaagcccgggaaacgggatcctgatcttgatcaaccgaggtcacaacatagtaaaagcgctattggtaatggtacaatcgcgcgtttacacttattcagaacgatttttttcaggagggcctacttgtcacacaggacggtaatgtcgtgcccggttattgagctgacacagcaacttattcgtcgcccctccctgagtccggatgacgcaggctgtcaggcattaatgattgaacgcctgcgtaaaatcggttttaccattgagcatatggattttggcgacacgcaaaatttttgggcatggcgtgggcgtggcgaaacgctggcgttcgccgggcatactgacgtcgtaccggctggcgatgtcgatcgctggatcaatccgccgtttgagcctacgattcgcgacggaatgttgttcggtcgcggcgcggcggatatgaaaggttcactggcggccatggtggtggctgctgaacgttttgttgcgcagcatcctcatcaccggggccgcctcgcatttttgattacctctgatgaggaagccagcgcaaaaaatggcaccgtaaaggtggttgaagcgctgatggcccgtaacgagcggctggattactgtctggtcggcgaaccttccagtactgaaattgtgggcgatgtcgtcaaaaacgggcgtcgcggttctctcacctgtaacctcactatccatggcgttcaggggcacgtcgcctatccgcatctggcggataaccctgttcatcgcgccgcgccttttcttaatgaactggtcgctatcgagtgggatcggggcaatgactttttcccggccaccagtatgcaggtagccaatatccaggcaggcaccggcagcaataatgtcattcccggcgaactgttcgtgcagtttaacttccgtttcagcacggaactgaccgatgagatgatcaaagagcgggtacatgcgctgcttgaaaagcatcagctacgctataccgtagactggtggctttccgggcagccgttcctgaccgcacgcggcaagctggtggacgcggtggtaaacgccattgagcactataatgaaattaaaccgcaattactgacgacgggcggtacgtccgacggacgttttatcgcccgtatgggagcgcaggtggtagaactggggccggtgaacgccaccattcataaaattaatgaatgtgtgaatgccgccgatctccagctactggcccgtatgtatcaacgcattatggaacagctcgtcgcccatcaccatcaccatcactaagattacttcgcattgcaatcagctacggactcaagcttacgtcaggtcatacgatgaaggcgataagtcgcgtaagttgctagcccacgcggctcaccttcacgggtgggcctttcttcgcgatccacatg

SEQ ID NO: 11 - DNA, 76 bp, synthetic construct
  source 1..76: mol_type = other DNA
ttcacagaaaagtgttgcccccttccatggcggaagggggacaaaggtgaatttgtcctactcaggagagcgttca

SEQ ID NO: 12 - DNA, 68 bp, synthetic construct
  source 1..68: mol_type = other DNA
tctgacgtacacagcaattttgcgttacctgttaatcgagattgaaacaccgaagaaaggcccacccg

SEQ ID NO: 13 - DNA, 72 bp, synthetic construct
  source 1..72: mol_type = other DNA
ttggtttcagtgaatcccgttatcagcagttttttgatgaggtgtagtctatttgtcctactcaggagagcg

SEQ ID NO: 14 - DNA, 68 bp, synthetic construct
  source 1..68: mol_type = other DNA
caatattttgccagccagtccatgcttatttcctcttaccggaacgctcacgaagaaaggcccacccg

SEQ ID NO: 15 - DNA, 65 bp, synthetic construct
  source 1..65: mol_type = other DNA
caatattttgccagccagtccatgcttatttcctcttaccggaacgctcaatttgtcctactcag

SEQ ID NO: 16 - DNA, 68 bp, synthetic construct
  source 1..68: mol_type = other DNA
ttggtttcagtgaatcccgttatcagcagttttttgatgaggtgtagtctcgaagaaaggcccacccg

SEQ ID NO: 17 - DNA, 71 bp, synthetic construct
  source 1..71: mol_type = other DNA
atgaaaaaaataatgctagtttttattacacttatattagttagtctaccgccgatcatattcaataaccc

SEQ ID NO: 18 - DNA, 70 bp, synthetic construct
  source 1..70: mol_type = other DNA
ttattcgattggattatctactttattactatatttcggataaagcgtggctagtgaacctcttcgaggg

SEQ ID NO: 19 - DNA, 71 bp, synthetic construct
  source 1..71: mol_type = other DNA
gataatgtattcacaggttgctccgggcttgaaaaagttaaatgacatccatttgtcctactcaggagagc

SEQ ID NO: 20 - DNA, 67 bp, synthetic construct
  source 1..67: mol_type = other DNA
aaaaggaactttttaccttttcgccttcccgtttcgttcaacttagtatacgaagaaaggcccaccc

SEQ ID NO: 21 - DNA, 71 bp, synthetic construct
  source 1..71: mol_type = other DNA
aggtagtacagggtttgtcagcataaagcctctcttacgagaggctttatgccgatcatattcaataaccc

SEQ ID NO: 22 - DNA, 70 bp, synthetic construct
  source 1..70: mol_type = other DNA
tcgctacactattcacaattccttttcgcgtcagcagaccctggaaaagcctagtgaacctcttcgaggg

SEQ ID NO: 23 - DNA, 71 bp, synthetic construct
  source 1..71: mol_type = other DNA
cggacaaaaaaatggcgcacgatgtgcgccattttatattgtgcgtcaaagccgatcatattcaataaccc

SEQ ID NO: 24 - DNA, 70 bp, synthetic construct
  source 1..70: mol_type = other DNA
aatacttgtaacgctacatggagattaactcaatctagagggtattaatactagtgaacctcttcgaggg

SEQ ID NO: 25 - DNA, 71 bp, synthetic construct
  source 1..71: mol_type = other DNA
gctttcgctgccttgattgtgtaccacgtgtcggtgaatcaatcgccggagccgatcatattcaataaccc

SEQ ID NO: 26 - DNA, 70 bp, synthetic construct
  source 1..70: mol_type = other DNA
acggtgagaaaccgtgggcaacagcccaataacatcaagttgtaattgatctagtgaacctcttcgaggg

SEQ ID NO: 27 - DNA, 1128 bp, Salmonella enterica
  source 1..1128: mol_type = other DNA
atgtcgtgcccggttattgagctgacacagcaacttattcgtcgcccctccctgagtccggatgacgcaggctgtcaggcattaatgattgaacgcctgcgtaaaatcggttttaccattgagcatatggattttggcgacacgcaaaatttttgggcatggcgtgggcgtggcgaaacgctggcgttcgccgggcatactgacgtcgtaccggctggcgatgtcgatcgctggatcaatccgccgtttgagcctacgattcgcgacggaatgttgttcggtcgcggcgcggcggatatgaaaggttcactggcggccatggtggtggctgctgaacgttttgttgcgcagcatcctcatcaccggggccgcctcgcatttttgattacctctgatgaggaagccagcgcaaaaaatggcaccgtaaaggtggttgaagcgctgatggcccgtaacgagcggctggattactgtctggtcggcgaaccttccagtactgaaattgtgggcgatgtcgtcaaaaacgggcgtcgcggttctctcacctgtaacctcactatccatggcgttcaggggcacgtcgcctatccgcatctggcggataaccctgttcatcgcgccgcgccttttcttaatgaactggtcgctatcgagtgggatcggggcaatgactttttcccggccaccagtatgcaggtagccaatatccaggcaggcaccggcagcaataatgtcattcccggcgaactgttcgtgcagtttaacttccgtttcagcacggaactgaccgatgagatgatcaaagagcgggtacatgcgctgcttgaaaagcatcagctacgctataccgtagactggtggctttccgggcagccgttcctgaccgcacgcggcaagctggtggacgcggtggtaaacgccattgagcactataatgaaattaaaccgcaattactgacgacgggcggtacgtccgacggacgttttatcgcccgtatgggagcgcaggtggtagaactggggccggtgaacgccaccattcataaaattaatgaatgtgtgaatgccgccgatctccagctactggcccgtatgtatcaacgcattatggaacagctcgtcgcctga

SEQ ID NO: 28 - DNA, 1428 bp, Salmonella enterica
  source 1..1428: mol_type = other DNA
atgaaaaaaaccacattagcaatgagtgcactggctctgagtttaggtttggcattgtcgcctctgtctgccacggcggctgaaacgtcctcttcagcaatgactgcccagcagatgccaagcctggcaccgatgctcgaaaaagtgatgccatcggtggtcagtattaatgttgaaggtagcaccacggtgaatacgccgcgtatgccgcgtaatttccagcagttctttggcgatgactccccgttctgccaggacggttctccgttccagaattctccgttctgccagggcggcggtaacggcggcaacggcggtcaacaacagaaattcatggcgctgggctccggcgtaattattgacgccgcgaagggctacgtcgtcaccaacaaccacgtggttgataacgccagcgtgattaaagtacagcttagcgatgggcgtaaattcgatgctaaagtggtgggcaaagatccgcgttctgatatcgcgctgattcaaattcagaatccgaagaacctgacggcgattaagctggcggactccgacgcgctgcgcgtgggggattataccgtcgctattggtaacccgtttggtctgggcgaaacggtgacgtcaggtatcgtttcggcgctggggcgtagcggcctgaacgtagaaaattacgagaactttattcagaccgacgccgcgattaaccgtggtaactccggcggcgcgctggtgaacctgaacggtgagctgatcggtattaacaccgcgattctggcgccggacggcggcaacatcggtatcggcttcgctatccccagtaacatggtgaaaaacctgacgtcgcagatggtggaatacggccaggtgaaacgcggcgaactggggatcatggggactgagctgaattccgaattggcgaaagcgatgaaagtcgacgcccagcgaggcgcgttcgtcagccaggtgatgccgaattcgtccgcggcgaaagcgggtatcaaagccggggatgtcattacctcgctgaacggtaaaccgatcagcagctttgcggcgctgcgcgctcaggtcggcactatgccggtcggcagcaaaatcagcctcggtctgctgcgtgaaggtaaagcgattacggtgaatctggaactgcagcagagcagccagagtcaggttgattccagcaccatcttcagcgggattgaaggcgctgaaatgagcaataaaggccaggataaaggcgttgtggtgagcagcgtgaaagcgaactcacccgccgcgcaaattggcctcaaaaaaggcgatgtgattatcggcgctaaccagcagccggtgaaaaatatcgccgagctgcgtaagattctcgacagcaagccgtcggttctggcgctgaatattcagcgtggtgatagttctatttatttgctgatgcagtaa

SEQ ID NO: 29 - DNA, 1590 bp, Listeria monocytogenes
  source 1..1590: mol_type = other DNA
atgaaaaaaataatgctagtttttattacacttatattagttagtctaccaattgcgcaacaaactgaagcaaaggatgcatctgcattcaataaagaaaattcaatttcatccatggcaccaccagcatctccgcctgcaagtcctaagacgccaatcgaaaagaaacacgcggatgaaatcgataagtatatacaaggattggactacaataaaaacaatgtattagtataccacggagatgcagtgacaaatgtgccgccaagaaaaggttacaaagatggaaatgaatatattgttgtggagaaaaagaagaaatccatcaatcaaaataatgcagacattcaagttgtgaatgcaatttcgagcctaacctatccaggtgctctcgtaaaagcgaattcggaattagtagaaaatcaaccagatgttctccctgtaaaacgtgattcattaacactcagcattgatttgccaggtatgactaatcaagacaataaaatcgttgtaaaaaatgccactaaatcaaacgttaacaacgcagtaaatacattagtggaaagatggaatgaaaaatatgctcaagcttatccaaatgtaagtgcaaaaattgattatgatgacgaaatggcttacagtgaatcacaattaattgcgaaatttggtacagcatttaaagctgtaaataatagcttgaatgtaaacttcggcgcaatcagtgaagggaaaatgcaagaagaagtcattagttttaaacaaatttactataacgtgaatgttaatgaacctacaagaccttccagatttttcggcaaagctgttactaaagagcagttgcaagcgcttggagtgaatgcagaaaatcctcctgcatatatctcaagtgtggcgtatggccgtcaagtttatttgaaattatcaactaattcccatagtactaaagtaaaagctgcttttgatgctgccgtaagcggaaaatctgtctcaggtgatgtagaactaacaaatatcatcaaaaattcttccttcaaagccgtaatttacggaggttccgcaaaagatgaagttcaaatcatcgacggcaacctcggagacttacgagatattttgaaaaaaggcgctacttttaatcgagaaacaccaggagttcccattgcttatacaacaaacttcctaaaagacaatgaattagctgttattaaaaacaactcagaatatattgaaacaacttcaaaagcttatacagatggaaaaattaacatcgatcactctggaggatacgttgctcaattcaacatttcttgggatgaagtaaattatgatcctgaaggtaacgaaattgttcaacataaaaactggagcgaaaacaataaaagtaagctagctcatttcacatcgtccatctatttgccaggtaacgcgagaaatattaatgtttacgctaaagaatgcactggtttagcttgggaatggtggagaacggtaattgatgaccggaacttaccacttgtgaaaaatagaaatatctccatctggggcaccacgctttatccgaaatatagtaataaagtagataatccaatcgaataa

SEQ ID NO: 30 - DNA, 85 bp, synthetic construct
  source 1..85: mol_type = other DNA
gcaggggtaaaagtgacctgacgcaatatttgtcttttcttgcttcttaataatgttgtcacaaaaagtgagggtgactacatgg

SEQ ID NO: 31 - DNA, 85 bp, synthetic construct
  source 1..85: mol_type = other DNA
cgccgcaaagtttgagcgaagtcaataaactctctacccattcagggcaatatctctcttgcaggtgaatgcaacgtcaagcgat

SEQ ID NO: 32 - DNA, 85 bp, synthetic construct
  source 1..85: mol_type = other DNA
tcagaagaagcaaaaagacactttaccgaagggtttaacattttttcgtgatactcatcaccatgacgcaaatgcgttgcataaa

SEQ ID NO: 33 - DNA, 85 bp, synthetic construct
  source 1..85: mol_type = other DNA
aaccgaggtcacaacatagtaaaagcgctattggtaatggtacaatcgcgcgtttacacttattcagaacgatttttttcaggag

SEQ ID NO: 34 - DNA, 54 bp, synthetic construct
  source 1..54: mol_type = other DNA
ggataaaagtgacctgacgcaatatttgtcttttcttgcttaataatgttgtca

SEQ ID NO: 35 - DNA, 35 bp, synthetic construct
  source 1..35: mol_type = other DNA
tgtaagtttatacataggcgagtactctgttatgg

SEQ ID NO: 36 - DNA, 74 bp, synthetic construct
  source 1..74: mol_type = other DNA
ttaaatttcctctcgtcaggccggaataactccctataatgcgccaccacactgatagtgctagtgtagatcac

SEQ ID NO: 37 - DNA, 58 bp, synthetic construct
  source 1..58: mol_type = other DNA
aaaattgatctgaatcaatattttgacaaaaattgatctgaatcaatatttactgagc

SEQ ID NO: 38 - DNA, 44 bp, synthetic construct
  source 1..44: mol_type = other DNA
gttaataaaatgttattgacagttaataaaatgttatactgagc

SEQ ID NO: 39 - DNA, 30 bp, synthetic construct
  source 1..30: mol_type = other DNA
ttagcacgttaattatctatcgtgtatatg